European Patent Specification EP 3 896 171 B1, published February 1, 2023. Title: METHODS AND SYSTEMS FOR PROCESSING POLYNUCLEOTIDES. Applicant: 10X GENOMICS, INC. Application PCT/US2017/068320. The sequence listing filed with the application follows.

SEQUENCE LISTING (64 sequences)

SEQ ID NO: 1 - DNA, 16 bp, Artificial Sequence
  Description of Artificial Sequence: Synthetic oligonucleotide
aaaaaaaaaaaaaaaa

SEQ ID NO: 2 - DNA, 11 bp, Artificial Sequence
  Description of Artificial Sequence: Synthetic oligonucleotide
aaaaaaaaaaa

SEQ ID NO: 3 - DNA, 11 bp, Artificial Sequence
  Description of Artificial Sequence: Synthetic oligonucleotide
ttttttttttt

SEQ ID NO: 4 - DNA, 78 bp, Artificial Sequence
  Description of Artificial Sequence: Synthetic oligonucleotide
  modified_base (23)..(28): a, c, t, or g
  modified_base (31)..(46): a, c, t, or g
  modified_base (78)..(78): a, c, t, or g
ctacacgacgctcttccgatctnnnnnntcnnnnnnnnnnnnnnnnttttttttttttttttttttttttttttttvn

SEQ ID NO: 5 - DNA, 46 bp, Artificial Sequence
  Description of Artificial Sequence: Synthetic oligonucleotide
  modified_base (23)..(28): a, c, t, or g
  modified_base (31)..(46): a, c, t, or g
ctacacgacgctcttccgatctnnnnnntcnnnnnnnnnnnnnnnn

SEQ ID NO: 6 - DNA, 52 bp, Artificial Sequence
  Description of Artificial Sequence: Synthetic oligonucleotide
  modified_base (23)..(38): a, c, t, or g
  modified_base (41)..(52): a, c, t, or g
ctacacgacgctcttccgatctnnnnnnnnnnnnnnnntcnnnnnnnnnnnn

SEQ ID NO: 7 - DNA, 44 bp, Artificial Sequence
  Description of Artificial Sequence: Synthetic oligonucleotide
  modified_base (23)..(36): a, c, t, or g
  modified_base (39)..(44): a, c, t, or g
ctacacgacgctcttccgatctnnnnnnnnnnnnnntcnnnnnn

SEQ ID NO: 8 - DNA, 53 bp, Artificial Sequence
  Description of Artificial Sequence: Synthetic primer
  modified_base (1)..(21): a, c, t, or g
  modified_base (53)..(53): a, c, t, or g
nnnnnnnnnnnnnnnnnnnnnttttttttttttttttttttttttttttttvn

SEQ ID NO: 9 - DNA, 52 bp, Artificial Sequence
  Description of Artificial Sequence: Synthetic primer
  modified_base (1)..(20): a, c, t, or g
  modified_base (52)..(52): a, c, t, or g
nnnnnnnnnnnnnnnnnnnnttttttttttttttttttttttttttttttvn

SEQ ID NO: 10 - DNA, 32 bp, Artificial Sequence
  Description of Artificial Sequence: Synthetic primer
  modified_base (32)..(32): a, c, t, or g
ttttttttttttttttttttttttttttttvn

SEQ ID NO: 11 - DNA, 114 bp, Artificial Sequence
  Description of Artificial Sequence: Synthetic polynucleotide
  modified_base (25)..(30): a, c, t, or g
  modified_base (33)..(38): a, c, t, or g
  modified_base (73)..(82): a, c, t, or g
  modified_base (114)..(114): a, c, t, or g
caagcagaagacggcatacgagatnnnnnngtnnnnnngtgactggagttcagacgtgtgctcttccgatctnnnnnnnnnnttttttttttttttttttttttttttttttvn

SEQ ID NO: 12 - DNA, 114 bp, Artificial Sequence
  Description of Artificial Sequence: Synthetic polynucleotide
  modified_base (25)..(30): a, c, t, or g
  modified_base (33)..(38): a, c, t, or g
  modified_base (73)..(82): a, c, t, or g
  modified_base (114)..(114): a, c, t, or g
caagcagaagacggcatacgagatnnnnnncannnnnngtgactggagttcagacgtgtgctcttccgatctnnnnnnnnnnttttttttttttttttttttttttttttttvn

SEQ ID NO: 13 - DNA, 114 bp, Artificial Sequence
  Description of Artificial Sequence: Synthetic polynucleotide
  modified_base (25)..(30): a, c, t, or g
  modified_base (33)..(38): a, c, t, or g
  modified_base (73)..(82): a, c, t, or g
  modified_base (114)..(114): a, c, t, or g
caagcagaagacggcatacgagatnnnnnnagnnnnnngtgactggagttcagacgtgtgctcttccgatctnnnnnnnnnnttttttttttttttttttttttttttttttvn

SEQ ID NO: 14 - DNA, 114 bp, Artificial Sequence
  Description of Artificial Sequence: Synthetic polynucleotide
  modified_base (25)..(30): a, c, t, or g
  modified_base (33)..(38): a, c, t, or g
  modified_base (73)..(82): a, c, t, or g
  modified_base (114)..(114): a, c, t, or g
caagcagaagacggcatacgagatnnnnnntcnnnnnngtgactggagttcagacgtgtgctcttccgatctnnnnnnnnnnttttttttttttttttttttttttttttttvn

SEQ ID NO: 15 - DNA, 78 bp, Artificial Sequence
  Description of Artificial Sequence: Synthetic oligonucleotide
  modified_base (23)..(28): a, c, t, or g
  modified_base (31)..(46): a, c, t, or g
  modified_base (78)..(78): a, c, t, or g
ctacacgacgctcttccgatctnnnnnngtnnnnnnnnnnnnnnnnttttttttttttttttttttttttttttttvn

SEQ ID NO: 16 - DNA, 78 bp, Artificial Sequence
  Description of Artificial Sequence: Synthetic oligonucleotide
  modified_base (23)..(28): a, c, t, or g
  modified_base (31)..(46): a, c, t, or g
  modified_base (78)..(78): a, c, t, or g
ctacacgacgctcttccgatctnnnnnncannnnnnnnnnnnnnnnttttttttttttttttttttttttttttttvn

SEQ ID NO: 17 - DNA, 78 bp, Artificial Sequence
  Description of Artificial Sequence: Synthetic oligonucleotide
  modified_base (23)..(28): a, c, t, or g
  modified_base (31)..(46): a, c, t, or g
  modified_base (78)..(78): a, c, t, or g
ctacacgacgctcttccgatctnnnnnnagnnnnnnnnnnnnnnnnttttttttttttttttttttttttttttttvn

SEQ ID NO: 18 - DNA, 118 bp, Artificial Sequence
  Description of Artificial Sequence: Synthetic polynucleotide
  modified_base (30)..(35): a, c, t, or g
  modified_base (38)..(43): a, c, t, or g
  modified_base (77)..(86): a, c, t, or g
  modified_base (118)..(118): a, c, t, or g
aatgatacggcgaccaccgagatctacacnnnnnngtnnnnnnacactctttccctacacgacgctcttccgatctnnnnnnnnnnttttttttttttttttttttttttttttttvn

SEQ ID NO: 19 - DNA, 78 bp, Artificial Sequence
  Description of Artificial Sequence: Synthetic oligonucleotide
  modified_base (23)..(28): a, c, t, or g
  modified_base (31)..(46): a, c, t, or g
  modified_base (78)..(78): a, c, t, or g
cagacgtgtgctcttccgatctnnnnnngtnnnnnnnnnnnnnnnnttttttttttttttttttttttttttttttvn

SEQ ID NO: 20 - DNA, 52 bp, Artificial Sequence
  Description of Artificial Sequence: Synthetic oligonucleotide
  modified_base (23)..(38): a, c, t, or g
  modified_base (41)..(52): a, c, t, or g
ctacacgacgctcttccgatctnnnnnnnnnnnnnnnngtnnnnnnnnnnnn

SEQ ID NO: 21 - DNA, 52 bp, Artificial Sequence
  Description of Artificial Sequence: Synthetic oligonucleotide
  modified_base (23)..(38): a, c, t, or g
  modified_base (41)..(52): a, c, t, or g
ctacacgacgctcttccgatctnnnnnnnnnnnnnnnncannnnnnnnnnnn

SEQ ID NO: 22 - DNA, 52 bp, Artificial Sequence
  Description of Artificial Sequence: Synthetic oligonucleotide
  modified_base (23)..(38): a, c, t, or g
  modified_base (41)..(52): a, c, t, or g
ctacacgacgctcttccgatctnnnnnnnnnnnnnnnnagnnnnnnnnnnnn

SEQ ID NO: 23 - DNA, 21 bp, Artificial Sequence
  Description of Artificial Sequence: Synthetic oligonucleotide
aaaaaaaaaaaaaaaaaaaaa

SEQ ID NO: 24 - DNA, 15 bp, Artificial Sequence
  Description of Artificial Sequence: Synthetic oligonucleotide
ctacacgacgctctt

SEQ ID NO: 25 - DNA, 28 bp, Artificial Sequence
  Description of Artificial Sequence: Synthetic oligonucleotide
  modified_base (23)..(28): a, c, t, or g
ctacacgacgctcttccgatctnnnnnn

SEQ ID NO: 26 - DNA, 22 bp, Artificial Sequence
  Description of Artificial Sequence: Synthetic oligonucleotide
  modified_base (3)..(8): a, c, t, or g
acnnnnnnagatcggaagagcg

SEQ ID NO: 27 - DNA, 50 bp, Artificial Sequence
  Description of Artificial Sequence: Synthetic oligonucleotide
  modified_base (3)..(18): a, c, t, or g
  modified_base (50)..(50): a, c, t, or g
gtnnnnnnnnnnnnnnnnttttttttttttttttttttttttttttttvn

SEQ ID NO: 28 - DNA, 41 bp, Artificial Sequence
  Description of Artificial Sequence: Synthetic oligonucleotide
  modified_base (3)..(18): a, c, t, or g
gtnnnnnnnnnnnnnnnntacgctagtttcgcgtacgaagc

SEQ ID NO: 29 - DNA, 69 bp, Artificial Sequence
  Description of Artificial Sequence: Synthetic oligonucleotide
  modified_base (23)..(28): a, c, t, or g
  modified_base (31)..(46): a, c, t, or g
ctacacgacgctcttccgatctnnnnnngtnnnnnnnnnnnnnnnntacgctagtttcgcgtacgaagc

SEQ ID NO: 30 - DNA, 80 bp, Artificial Sequence
  Description of Artificial Sequence: Synthetic oligonucleotide
  modified_base (23)..(48): a, c, t, or g
  modified_base (80)..(80): a, c, t, or g
ctacacgacgctcttccgatctnnnnnnnnnnnnnnnnnnnnnnnnnnttttttttttttttttttttttttttttttvn

SEQ ID NO: 31 - DNA, 70 bp, Artificial Sequence
  Description of Artificial Sequence: Synthetic oligonucleotide
  modified_base (23)..(48): a, c, t, or g
ctacacgacgctcttccgatctnnnnnnnnnnnnnnnnnnnnnnnnnnacgctagtttcgcgtacgaagc

SEQ ID NO: 32 - DNA, 15 bp, Artificial Sequence
  Description of Artificial Sequence: Synthetic oligonucleotide
gtcagatgtgtataa

SEQ ID NO: 33 - DNA, 80 bp, Artificial Sequence
  Description of Artificial Sequence: Synthetic oligonucleotide
  modified_base (23)..(29): a, c, t, or g
  modified_base (32)..(48): a, c, t, or g
  modified_base (80)..(80): a, c, t, or g
ctacacgacgctcttccgatctnnnnnnngtnnnnnnnnnnnnnnnnnttttttttttttttttttttttttttttttvn

SEQ ID NO: 34 - DNA, 80 bp, Artificial Sequence
  Description of Artificial Sequence: Synthetic oligonucleotide
  modified_base (23)..(29): a, c, t, or g
  modified_base (32)..(48): a, c, t, or g
  modified_base (80)..(80): a, c, t, or g
ctacacgacgctcttccgatctnnnnnnncannnnnnnnnnnnnnnnnttttttttttttttttttttttttttttttvn

SEQ ID NO: 35 - DNA, 80 bp, Artificial Sequence
  Description of Artificial Sequence: Synthetic oligonucleotide
  modified_base (23)..(29): a, c, t, or g
  modified_base (32)..(48): a, c, t, or g
  modified_base (80)..(80): a, c, t, or g
ctacacgacgctcttccgatctnnnnnnnagnnnnnnnnnnnnnnnnnttttttttttttttttttttttttttttttvn

SEQ ID NO: 36 - DNA, 80 bp, Artificial Sequence
  Description of Artificial Sequence: Synthetic oligonucleotide
  modified_base (23)..(29): a, c, t, or g
  modified_base (32)..(48): a, c, t, or g
  modified_base (80)..(80): a, c, t, or g
ctacacgacgctcttccgatctnnnnnnntcnnnnnnnnnnnnnnnnnttttttttttttttttttttttttttttttvn

SEQ ID NO: 37 - DNA, 70 bp, Artificial Sequence
  Description of Artificial Sequence: Synthetic oligonucleotide
  modified_base (23)..(29): a, c, t, or g
  modified_base (32)..(48): a, c, t, or g
gtcagatgtgtataagagacagnnnnnnngtnnnnnnnnnnnnnnnnngcttcgtacgcgaaactagcgt

SEQ ID NO: 38 - DNA, 60 bp, Artificial Sequence
  Description of Artificial Sequence: Synthetic oligonucleotide
  Description of Combined DNA/RNA Molecule: Synthetic oligonucleotide
  modified_base (23)..(47): a, c, t, or g
ctacacgacgctcttccgatctnnnnnnnnnnnnnnnnnnnnnnnnntttcttatatggg

SEQ ID NO: 39 - DNA, 43 bp, Artificial Sequence
  Description of Artificial Sequence: Synthetic oligonucleotide
caactttagcggtccaaggtgcagtcagatcccatataagaaa

SEQ ID NO: 40 - protein, 6 aa, Artificial Sequence
  Description of Artificial Sequence: Synthetic 6xHis tag
HHHHHH

SEQ ID NO: 41 - DNA, 61 bp, Artificial Sequence
  Description of Artificial Sequence: Synthetic oligonucleotide
  modified_base (35)..(40): a, c, t, or g
  modified_base (43)..(48): a, c, t, or g
agatcggaagagcacacgtctgaactccagtcacnnnnnnacnnnnnnatctcgtatgccg

SEQ ID NO: 42 - DNA, 61 bp, Artificial Sequence
  Description of Artificial Sequence: Synthetic oligonucleotide
  modified_base (35)..(40): a, c, t, or g
  modified_base (43)..(48): a, c, t, or g
agatcggaagagcacacgtctgaactccagtcacnnnnnntgnnnnnnatctcgtatgccg

SEQ ID NO: 43 - DNA, 61 bp, Artificial Sequence
  Description of Artificial Sequence: Synthetic oligonucleotide
  modified_base (35)..(40): a, c, t, or g
  modified_base (43)..(48): a, c, t, or g
agatcggaagagcacacgtctgaactccagtcacnnnnnnctnnnnnnatctcgtatgccg

SEQ ID NO: 44 - DNA, 61 bp, Artificial Sequence
  Description of Artificial Sequence: Synthetic oligonucleotide
  modified_base (35)..(40): a, c, t, or g
  modified_base (43)..(48): a, c, t, or g
agatcggaagagcacacgtctgaactccagtcacnnnnnngannnnnnatctcgtatgccg

SEQ ID NO: 45 - DNA, 28 bp, Artificial Sequence
  Description of Artificial Sequence: Synthetic oligonucleotide
  modified_base (1)..(6): a, c, t, or g
  modified_base (9)..(14): a, c, t, or g
nnnnnnacnnnnnnagatcggaagagcg

SEQ ID NO: 46 - DNA, 28 bp, Artificial Sequence
  Description of Artificial Sequence: Synthetic oligonucleotide
  modified_base (1)..(6): a, c, t, or g
  modified_base (9)..(14): a, c, t, or g
nnnnnntgnnnnnnagatcggaagagcg

SEQ ID NO: 47 - DNA, 28 bp, Artificial Sequence
  Description of Artificial Sequence: Synthetic oligonucleotide
  modified_base (1)..(6): a, c, t, or g
  modified_base (9)..(14): a, c, t, or g
nnnnnnctnnnnnnagatcggaagagcg

SEQ ID NO: 48 - DNA, 28 bp, Artificial Sequence
  Description of Artificial Sequence: Synthetic oligonucleotide
  modified_base (1)..(6): a, c, t, or g
  modified_base (9)..(14): a, c, t, or g
nnnnnngannnnnnagatcggaagagcg

SEQ ID NO: 49 - DNA, 62 bp, Artificial Sequence
  Description of Artificial Sequence: Synthetic oligonucleotide
  modified_base (34)..(39): a, c, t, or g
  modified_base (42)..(47): a, c, t, or g
agatcggaagagcgtcgtgtagggaaagagtgtnnnnnnacnnnnnngtgtagatctcggtg

SEQ ID NO: 50 - DNA, 27 bp, Artificial Sequence
  Description of Artificial Sequence: Synthetic oligonucleotide
  modified_base (1)..(6): a, c, t, or g
  modified_base (9)..(14): a, c, t, or g
nnnnnnacnnnnnnagatcggaagagc

SEQ ID NO: 51 - DNA, 14 bp, Artificial Sequence
  Description of Artificial Sequence: Synthetic oligonucleotide
agatcggaagagcg

SEQ ID NO: 52 - DNA, 30 bp, Artificial Sequence
  Description of Artificial Sequence: Synthetic oligonucleotide
  modified_base (1)..(7): a, c, t, or g
  modified_base (10)..(16): a, c, t, or g
nnnnnnnacnnnnnnnagatcggaagagcg

SEQ ID NO: 53 - DNA, 30 bp, Artificial Sequence
  Description of Artificial Sequence: Synthetic oligonucleotide
  modified_base (1)..(7): a, c, t, or g
  modified_base (10)..(16): a, c, t, or g
nnnnnnntgnnnnnnnagatcggaagagcg

SEQ ID NO: 54 - DNA, 30 bp, Artificial Sequence
  Description of Artificial Sequence: Synthetic oligonucleotide
  modified_base (1)..(7): a, c, t, or g
  modified_base (10)..(16): a, c, t, or g
nnnnnnnctnnnnnnnagatcggaagagcg

SEQ ID NO: 55 - DNA, 30 bp, Artificial Sequence
  Description of Artificial Sequence: Synthetic oligonucleotide
  modified_base (1)..(7): a, c, t, or g
  modified_base (10)..(16): a, c, t, or g
nnnnnnngannnnnnnagatcggaagagcg

SEQ ID NO: 56 - DNA, 31 bp, Artificial Sequence
  Description of Artificial Sequence: Synthetic oligonucleotide
  modified_base (1)..(7): a, c, t, or g
  modified_base (10)..(16): a, c, t, or g
nnnnnnnacnnnnnnnctgtctcttatacac

SEQ ID NO: 57 - DNA, 24 bp, Artificial Sequence
  Description of Artificial Sequence: Synthetic oligonucleotide
caactttagcggtccaaggtgcat

SEQ ID NO: 58 - DNA, 88 bp, Artificial Sequence
  Description of Artificial Sequence: Synthetic oligonucleotide
  modified_base (56)..(65): a, c, t, or g
caccttggaccgctaaagttggtgactggagttcagacgtgtgctcttccgatctnnnnnnnnnncagatttgaccccatataagaaa

SEQ ID NO: 59 - DNA, 20 bp, Artificial Sequence
  Description of Artificial Sequence: Synthetic oligonucleotide
aaaaaaaaaaaaaaaaaaaa

SEQ ID NO: 60 - DNA, 10 bp, Artificial Sequence
  Description of Artificial Sequence: Synthetic oligonucleotide
atcctagcaa

SEQ ID NO: 61 - DNA, 12 bp, Artificial Sequence
  Description of Artificial Sequence: Synthetic oligonucleotide
tgatcctagcaa

SEQ ID NO: 62 - protein, 9 aa, Artificial Sequence
  Description of Artificial Sequence: Synthetic peptide
EGALIYWPN

SEQ ID NO: 63 - protein, 8 aa, Artificial Sequence
  Description of Artificial Sequence: Synthetic peptide
AHMRDSQQ

SEQ ID NO: 64 - protein, 9 aa, Epstein-Barr virus
GLCTLVAML